European Patent Application EP 4 163 292 A1, published April 12, 2023. Title: Rhodopsin mutants. Applicant: SHIZUOKA PREFECTURE PUBLIC UNIVERSITY CORPORATION. The sequence listing filed with the application follows.

SEQUENCE LISTING (13 sequences)

SEQ ID NO: 1 - DNA, 24 bp, synthetic construct
  misc_feature 1..24: note = dR_colony_F3 forward
  source 1..24: mol_type = other DNA
cgtattgtacacggccgcataatc

SEQ ID NO: 2 - DNA, 25 bp, synthetic construct
  misc_feature 1..25: note = dR_colony_R3 reverse
  source 1..25: mol_type = other DNA
tatgctagttattgctcagcggtgg

SEQ ID NO: 3 - protein, 256 aa, Rhodobacterales bacterium
MTILSKKGFKVALATVAAGILPASAHAATLQPNDFVGISFWLISMALVAATVFFFMEAGRVSAKWRTSLTVSGLVTLIAAVHYFYMRDVWVATGETPTVYRYIDWLLTVPLLMVEFYLILRAIGAVSAGIFWRLLIGSLVMLIAGYLGEAGYINVWLGFVIGMAGWIYILYEIFAGEAGKASAESAPEAVQSAFNTMRLIVTVGWAIYPLGYFLGYMGGAVDAATLNVIYNVADFVNKIAFGLVIWNVAVTESESK

SEQ ID NO: 4 - protein, 256 aa, synthetic construct
  REGION 1..256: note = OP27 mutant
  SITE 31: note = misc_feature - Xaa can be any naturally occurring amino acid
  SITE 128: note = misc_feature - Xaa can be any naturally occurring amino acid
MTILSKKGFKVALATVAAGILPASAHAATLXPNDYVGISFWLISMALIAATAFFFIETTRVEGKWKTSLTVSGLVTLVAAVHYFYMRDVWVSTGESPTVYRYIDWLITVPLLMVEFYLILRAITKVSXGIFWRLMIGTVVMLVGGYAGEIGYISATLGFIIGMLGWAYILYEIFAGEASKVAADEAPASVQSAFSTMRWIVTIGWAIYPLGYFMGYMNGAVSDEALNIIYNFADVWNKIAFGVIIWNVAVTESESK

SEQ ID NO: 5 - protein, 257 aa, synthetic construct
  REGION 1..257: note = OP27-A10
MMTILSKKGFKVALATVAAGILPASAHAATLQPNDFVGISFWLISMAMVASTVFFFMEANRVSAKWRTSLTVAGLVTLIAAVHYFYMRDVWVATGETPTVYRYIDWLLTVPLQMIEFYLILAAVGAVSAGIFWRLLIGTLVMLIAGYLGEAGYINVTVGFVIGMAGWIYILYEIFAGEAGKASAESASEAVKSAFNAMRWIVTVGWAIYPLGYFLGYMTGAVDDATLNVIYNLADFVNKIAFGLVIWNVAVTESESK

SEQ ID NO: 6 - protein, 257 aa, synthetic construct
  REGION 1..257: note = OP27-A20
MMTILSKKGFKVALATVAAGILPASAHAATLQPDDFVGISFWLISMALVASTVFFFMETQRVSAKWKTSLTVSGLVTLIAAVHYFYMRDVWVATGETPTVYRYIDWLLTVPLLMIEFYLILRAIGAVSAGIFWRLLIGTLVMLIGGYLGEAGYINVTVGFVIGMAGWVYILYEIFAGEAGKAAADEASESVKSAYNAMRWIVTVGWAIYPLGYFLGYMTGAVDDATLNIIYNLADVVNKIAFGLIIWNVAVTESESK

SEQ ID NO: 7 - protein, 257 aa, synthetic construct
  REGION 1..257: note = OP27-A110
MMTILSKKGFKVALATVAAGILPASAHAATLQPDDFVGISFWLISMALVASTAFFFMETQRVSAKWKTSLTVSGLVTLIAAVHYFYMRDVWVATGETPTVYRYIDWLITVPLLMIEFYLILRAITNVSAGIFWRLMIGTLVMLIGGYLGEAGYINVTVGFVIGMAGWAYILYEIFAGEAGKVAADEAPESVKSAYSTMRWIVTIGWAIYPLGYFLGYMAGAVDDATLNIIYNLADVLNKIAFGVIIWNVAVTESESK

SEQ ID NO: 8 - protein, 257 aa, synthetic construct
  REGION 1..257: note = OP27 mutant2
  SITE 1: note = misc_feature - Xaa can be any naturally occurring amino acid
  SITE 32: note = misc_feature - Xaa can be any naturally occurring amino acid
  SITE 34: note = misc_feature - Xaa can be any naturally occurring amino acid
  SITE 36: note = misc_feature - Xaa can be any naturally occurring amino acid
  REGION 48..49: note = misc_feature - Xaa can be any naturally occurring amino acid
  SITE 51: note = misc_feature - Xaa can be any naturally occurring amino acid
  SITE 53: note = misc_feature - Xaa can be any naturally occurring amino acid
  SITE 57: note = misc_feature - Xaa can be any naturally occurring amino acid
  REGION 59..60: note = misc_feature - Xaa can be any naturally occurring amino acid
  REGION 63..64: note = misc_feature - Xaa can be any naturally occurring amino acid
  SITE 67: note = misc_feature - Xaa can be any naturally occurring amino acid
  SITE 73: note = misc_feature - Xaa can be any naturally occurring amino acid
  SITE 79: note = misc_feature - Xaa can be any naturally occurring amino acid
  SITE 93: note = misc_feature - Xaa can be any naturally occurring amino acid
  SITE 97: note = misc_feature - Xaa can be any naturally occurring amino acid
  SITE 108: note = misc_feature - Xaa can be any naturally occurring amino acid
  SITE 113: note = misc_feature - Xaa can be any naturally occurring amino acid
  SITE 115: note = misc_feature - Xaa can be any naturally occurring amino acid
  SITE 122: note = misc_feature - Xaa can be any naturally occurring amino acid
  REGION 124..126: note = misc_feature - Xaa can be any naturally occurring amino acid
  SITE 129: note = misc_feature - Xaa can be any naturally occurring amino acid
  SITE 136: note = misc_feature - Xaa can be any naturally occurring amino acid
  SITE 140: note = misc_feature - Xaa can be any naturally occurring amino acid
  REGION 144..145: note = misc_feature - Xaa can be any naturally occurring amino acid
  SITE 148: note = misc_feature - Xaa can be any naturally occurring amino acid
  SITE 151: note = misc_feature - Xaa can be any naturally occurring amino acid
  REGION 155..156: note = misc_feature - Xaa can be any naturally occurring amino acid
  SITE 158: note = misc_feature - Xaa can be any naturally occurring amino acid
  SITE 161: note = misc_feature - Xaa can be any naturally occurring amino acid
  SITE 165: note = misc_feature - Xaa can be any naturally occurring amino acid
  SITE 168: note = misc_feature - Xaa can be any naturally occurring amino acid
  SITE 180: note = misc_feature - Xaa can be any naturally occurring amino acid
  REGION 182..183: note = misc_feature - Xaa can be any naturally occurring amino acid
  REGION 185..186: note = misc_feature - Xaa can be any naturally occurring amino acid
  REGION 188..190: note = misc_feature - Xaa can be any naturally occurring amino acid
  SITE 192: note = misc_feature - Xaa can be any naturally occurring amino acid
  REGION 195..197: note = misc_feature - Xaa can be any naturally occurring amino acid
  SITE 204: note = misc_feature - Xaa can be any naturally occurring amino acid
  SITE 211: note = misc_feature - Xaa can be any naturally occurring amino acid
  SITE 215: note = misc_feature - Xaa can be any naturally occurring amino acid
  SITE 219: note = misc_feature - Xaa can be any naturally occurring amino acid
  SITE 223: note = misc_feature - Xaa can be any naturally occurring amino acid
  REGION 225..226: note = misc_feature - Xaa can be any naturally occurring amino acid
  SITE 229: note = misc_feature - Xaa can be any naturally occurring amino acid
  SITE 233: note = misc_feature - Xaa can be any naturally occurring amino acid
  REGION 236..237: note = misc_feature - Xaa can be any naturally occurring amino acid
  REGION 244..245: note = misc_feature - Xaa can be any naturally occurring amino acid
  REGION 43: note = misc_feature - Xaa can be any naturally occurring amino acid
  REGION 139: note = misc_feature - Xaa can be any naturally occurring amino acid
  REGION 157: note = misc_feature - Xaa can be any naturally occurring amino acid
  REGION 200: note = misc_feature - Xaa can be any naturally occurring amino acid
  REGION 224: note = misc_feature - Xaa can be any naturally occurring amino acid
XMTILSKKGFKVALATVAAGILPASAHAATLXPXDXVGISFWLISMAXXAXTXFFFXEXXRVXXKWXTSLTVXGLVTLXAAVHYFYMRDVWVXTGEXPTVYRYIDWLXTVPLXMXEFYLILXAXXXVSXGIFWRLXIGTXVMLXXGYXGEXGYIXXTXGFXIGMXGWXYILYEIFAGEAXKXXAXXAXXXVXSAXXXMRWIVTXGWAIYPXGYFXGYMXGAVXDXXLNXIYNXADXXNKIAFGXXIWNVAVTESESK

SEQ ID NO: 9 - protein, 250 aa, synthetic construct
  REGION 1..250: note = dR
MCCAALAPPMAATVGPESIWLWIGTIGMTLGTLYFVGRGRGVRDRKMQEFYIITIFITTIAAAMYFAMATGFGVTEVMVGDEALTIYWARYADWLFTTPLLLLDLSLLAGANRNTIATLIGLDVFMIGTGAIAALSSTPGTRIAWWAISTGALLALLYVLVGTLSENARNRAPEVASLFGRLRNLVIALWFLYPVVWILGTEGTFGILPLYWETAAFMVLDLSAKVGFGVILLQSRSVLERVATPTAAPT

SEQ ID NO: 10 - protein, 250 aa, synthetic construct
  REGION 1..250: note = E104
MCCAALAPPMAATVGPESIWLWIGTIGMTLGTLYFVGRGRGVRDRKMQEFYIITIFITTIAAAMYFAMATGFGVTEVMVGDEALTIYWARYADWLFTTPLLLLDLSLLAGANRNTIATLIGLDVLMIGTGAIAALSSTPGTHIAWWAISTGALLALLYVLVGTLSENARNRAPEVASLFGRLRNLVIALWFLYPVVWILGTEGTFGILPLYWETAAFMVLDLSAKVGFGVILLQSRSVLERVATPTAAPT

SEQ ID NO: 11 - protein, 250 aa, synthetic construct
  REGION 1..250: note = E59
MCCAALAPPMAATVGPESIWLWIGTIGMTLGTLYFVGRGRGVRDRKMQEFYIITIFITTIAAAMYFAMATGFGVTEVMVGDEALTIYWARYADWLFTTPLLLLDLSLLAGANRNTIATLIGLDVFMIGTGAIAALSSTPGTRIAWWAISTGALLALLYVLVGTLSENARNRAPEVASLFGRLRNLVIALWFLYPVVWILGTEGTFGILPLYWETAAFMVLDLSAKVGFGVILLQSRSVLERAATPTAAPT

SEQ ID NO: 12 - protein, 250 aa, synthetic construct
  REGION 1..250: note = dR mutant
  SITE 125: note = misc_feature - Xaa can be any naturally occurring amino acid
  SITE 142: note = misc_feature - Xaa can be any naturally occurring amino acid
  SITE 242: note = misc_feature - Xaa can be any naturally occurring amino acid
MCCAALAPPMAATVGPESIWLWIGTIGMTLGTLYFVGRGRGVRDRKMQEFYIITIFITTIAAAMYFAMATGFGVTEVMVGDEALTIYWARYADWLFTTPLLLLDLSLLAGANRNTIATLIGLDVXMIGTGAIAALSSTPGTXIAWWAISTGALLALLYVLVGTLSENARNRAPEVASLFGRLRNLVIALWFLYPVVWILGTEGTFGILPLYWETAAFMVLDLSAKVGFGVILLQSRSVLERXATPTAAPT

SEQ ID NO: 13 - protein, 257 aa, synthetic construct
MMTILSKKGFKVALATVAAGILPASAHAATLQPNDFVGISFWIISMAMVAATVFFFMEAGRVSAKWRTSLTVAGLVTLIAAVHYFYMRDVWVATGETPTVYRYIDWLLTVPLQMVEFYLILAAVGAVSAGIFWRLLIGSLVMLIAGYLGEAGYINVWLGFVIGMAGWIYILYEIFAGEAGKASAESAPEAVQSAFNTMRLIVTVGWAIYPLGYFLGYMGGAVDAATLNVIYNVADFVNKIAFGLVIWNVAVTESESK